European Patent Application EP 4 353 823 A1, published April 17, 2024. Title: INHIBITORS OF MICRO-RNA 22. Applicant: Resalis Therapeutic srl. The sequence listing filed with the application follows.

SEQUENCE LISTING (27 sequences)

SEQ ID NO: 1 - RNA, 22 nt, Homo sapiens
  source 1..22: mol_type = genomic RNA
aagctgccagttgaagaactgt

SEQ ID NO: 2 - skipped

SEQ ID NO: 3 - DNA, 15 bp, synthetic construct
  misc_feature 1..15: note = Synthetic Nucleic Acid
  source 1..15: mol_type = other DNA
cttcaactggcagct

SEQ ID NO: 4 - DNA, 16 bp, synthetic construct
  misc_feature 1..16: note = Synthetic Nucleic Acid
  source 1..16: mol_type = other DNA
tcttcaactggcagct

SEQ ID NO: 5 - DNA, 17 bp, synthetic construct
  misc_feature 1..17: note = Synthetic Nucleic Acid
  source 1..17: mol_type = other DNA
ttcttcaactggcagct

SEQ ID NO: 6 - DNA, 18 bp, synthetic construct
  misc_feature 1..18: note = Synthetic Nucleic Acid
  source 1..18: mol_type = other DNA
gttcttcaactggcagct

SEQ ID NO: 7 - DNA, 15 bp, synthetic construct
  misc_feature 1..15: note = Synthetic Nucleic Acid
  source 1..15: mol_type = other DNA
cttcaactggcagct

SEQ ID NO: 8 - DNA, 15 bp, synthetic construct
  misc_feature 1..15: note = Synthetic Nucleic Acid
  source 1..15: mol_type = other DNA
cttcaactggcagct

SEQ ID NO: 9 - DNA, 16 bp, synthetic construct
  misc_feature 1..16: note = Synthetic Nucleic Acid
  source 1..16: mol_type = other DNA
tcttcaactggcagct

SEQ ID NO: 10 - DNA, 16 bp, synthetic construct
  misc_feature 1..16: note = Synthetic Nucleic Acid
  source 1..16: mol_type = other DNA
tcttcaactggcagct

SEQ ID NO: 11 - DNA, 16 bp, synthetic construct
  misc_feature 1..16: note = Synthetic Nucleic Acid
  source 1..16: mol_type = other DNA
tcttcaactggcagct

SEQ ID NO: 12 - DNA, 17 bp, synthetic construct
  misc_feature 1..17: note = Synthetic Nucleic Acid
  source 1..17: mol_type = other DNA
ttcttcaactggcagct

SEQ ID NO: 13 - DNA, 18 bp, synthetic construct
  misc_feature 1..18: note = Synthetic Nucleic Acid
  source 1..18: mol_type = other DNA
gttcttcaactggcagct

SEQ ID NO: 14 - DNA, 16 bp, synthetic construct
  misc_feature 1..16: note = Synthetic Nucleic Acid
  source 1..16: mol_type = other DNA
cgaatagttagtagcg

SEQ ID NO: 15 - DNA, 16 bp, synthetic construct
  misc_feature 1..16: note = Synthetic Nucleic Acid
  source 1..16: mol_type = other DNA
cgaatagttagtagcg

SEQ ID NO: 16 - DNA, 18 bp, synthetic construct
  source 1..18: mol_type = other DNA
gttcttcaactggcagct

SEQ ID NO: 17 - DNA, 18 bp, synthetic construct
  source 1..18: mol_type = other DNA
gttcttcaactggcagct

SEQ ID NO: 18 - DNA, 18 bp, synthetic construct
  source 1..18: mol_type = other DNA
gttcttcaactggcagct

SEQ ID NO: 19 - DNA, 18 bp, synthetic construct
  source 1..18: mol_type = other DNA
gttcttcaactggcagct

SEQ ID NO: 20 - DNA, 18 bp, synthetic construct
  source 1..18: mol_type = other DNA
gttcttcaactggcagct

SEQ ID NO: 21 - DNA, 15 bp, synthetic construct
  source 1..15: mol_type = other DNA
cttcaactggcagct

SEQ ID NO: 22 - DNA, 35 bp, synthetic construct
  source 1..35: mol_type = other DNA
ctcgagacagttcttcaactggcagcttgcggccg

SEQ ID NO: 23 - DNA, 29 bp, synthetic construct
  source 1..29: mol_type = other DNA
ggccgcaagctgccagttgaagaactgtc

SEQ ID NO: 24 - DNA, 24 bp, synthetic construct
  source 1..24: mol_type = other DNA
ctattgtcgagggagctaagaagt

SEQ ID NO: 25 - DNA, 24 bp, synthetic construct
  source 1..24: mol_type = other DNA
cgcaagctgccagttgaagaactg

SEQ ID NO: 26 - DNA, 24 bp, synthetic construct
  source 1..24: mol_type = other DNA
ctattgtcgagggagctaagaagt

SEQ ID NO: 27 - DNA, 21 bp, synthetic construct
  source 1..21: mol_type = other DNA
gcgtcagacaaaccctaacca